European Patent Application EP 4 725 970 A1, published April 15, 2026. Title: 抗GPRC5D/BCMA/CD3三特异性抗体的制备及其用途. Applicant: 信达生物制药（苏州）有限公司. The sequence listing filed with the application follows.

SEQUENCE LISTING (116 sequences)

SEQ ID NO: 1 - protein, 215 aa, artificial sequence
QAVVTQEPSLTVSPGGTVTLTCRSSTGAVTTSNYANWVQKKPGQAPRGLIGGTNKRAPGVPARFSGSLLGDKAALTLLGAQPEDEAEYYCALWYSNLWVFGQGTKLTVLGQPKAAPSVTLFPPSSEELQANKATLVCLISDFYPGAVTVAWKADSSPVKAGVETTTPSKQSNNKYAASSYLSLTPEQWKSHRSYSCQVTHEGSTVEKTVAPTECS

SEQ ID NO: 2 - protein, 213 aa, artificial sequence
DIQMTQSPSSLSASVGDRVTITCRASQSISRYLNWYQDKPGKAPKLLIYAASSLQSGVPSRFSGSGSGTDFTLTISSLQPEDFATYYCQQKYFDITFGGGTKVEIKRTVAAPSVFIFPPSDECLKSGTASVVCLLNNFYPREAKVQWKVDNALQSGNSQESVTEQDSKDSTYSLSSTLTLSKADYEKHKVYACEVTHQGLSSPVTKSFNRGES

SEQ ID NO: 3 - protein, 687 aa, artificial sequence
QLQLQESGPGLVKPSETLSLTCTVSGGSISSSSYYWTWIRKPPGKGLEWIGSISIAGSTYYNPSLKSRVTISVDTSKNQFSLKLSSVTAADTAVYYCARDRGDQILDVWGQGTLVTVSSASTKGPSVCPLAPSSKSTSGGTAALGCLVKDYFPEPVTVSWNSGALTSGVHTFPAVLQSSGLYSLSSVVTVPSSSLGTQTYICNVNHKPSNTKVDKKVEPKSSGGGGSGGGGSEVQLVESGGGLVQPGGSLKLSCAASGFTFNTYAMNWVRDASGKGLEWVGRIRSKYNNYATYYADSVKDRFTISRDDSKSTLYLQMNSLKTEDTAVYYCARHGNFGQSYVSWFAYWGQGTTVTVSSASTKGPSVFPLAPSSKSTSGGTAALGCLVKDYFPEPVTVSWNSGALTSGVHTFPAVLQSSGLYSLSSVVTVPSSSLGTQTYICNVNHKPSNTKVDKKVEPKSCDKTHTCPPCPAPEAAGGPSVFLFPPKPKDTLMISRTPEVTCVVVDVSHEDPEVKFNWYVDGVEVHNAKTKPREEQYNSTYRVVSVLTVLHQDWLNGKEYKCKVSNKALPAPIEKTISKAKGQPREPQVYTLPPSRDELTKNQVSLSCAVKGFYPSDIAVEWESNGQPENNYKTTPPVLDSDGSFFLVSKLTVDKSRWQQGNVFSCSVMHEALHNHYTQKSLSLSPGK

SEQ ID NO: 4 - protein, 218 aa, artificial sequence
DIVMTQSPDSLAVSLGERATINCRASESVDSYGITFMNWYQQKPGQPPKLLIYAASNQGSGVPDRFSGSGSGTDFTLTISSLQAEDVAVYYCQQSKEVPWTFGQGTKLEIKRTVAAPSVFIFPPSDEQLKSGTASVVCLLNNFYPREAKVQWKVDNALQSGNSQESVTEQDSKDSTYSLSSTLTLSKADYEKHKVYACEVTHQGLSSPVTKSFNRGEC

SEQ ID NO: 5 - protein, 450 aa, artificial sequence
QVQLVQSGAEVKKPGASVKVSCKASGYTFIGYVMHWVRQAPGQGLEWMGYINPYNDVSQHQGKFKGRVTMTSDTSTSTVYMELSSLRSEDTAVYYCAREGRLGLRVLAYWGQGTLVTVSSASTKGPSVFPLAPSSKSTSGGTAALGCLVKDYFPEPVTVSWNSGALTSGVHTFPAVLQSSGLYSLSSVVTVPSSSLGTQTYICNVNHKPSNTKVDKKVEPKSCDKTHTCPPCPAPEAAGGPSVFLFPPKPKDTLMISRTPEVTCVVVDVSHEDPEVKFNWYVDGVEVHNAKTKPREEQYNSTYRVVSVLTVLHQDWLNGKEYKCKVSNKALPAPIEKTISKAKGQPREPQVYTLPPSRDELTKNQVSLWCLVKGFYPSDIAVEWESNGQPENNYKTTPPVLDSDGSFFLYSKLTVDKSRWQQGNVFSCSVMHEALHNHYTQKSLSLSPGK

SEQ ID NO: 6 - protein, 687 aa, artificial sequence
QLQLQESGPGLVKPSETLSLTCTVSGGSISSSSYYWTWIRKPPGKGLEWIGSISIAGSTYYNPSLKSRVTISVDTSKNQFSLKLSSVTAADTAVYYCARDRGDQILDVWGQGTLVTVSSASTKGPSVCPLAPSSKSTSGGTAALGCLVKDYFPEPVTVSWNSGALTSGVHTFPAVLQSSGLYSLSSVVTVPSSSLGTQTYICNVNHKPSNTKVDKKVEPKSSGGGGSGGGGSEVQLVESGGGLVQPGGSLKLSCAASGFTFNTYAMNWVRDASGKGLEWVGRIRSKYNNYATYYADSVKDRFTISRDDSKSTLYLQMNSLKTEDTAVYYCARHYNFGQSYVSWFAYWGQGTTVTVSSASTKGPSVFPLAPSSKSTSGGTAALGCLVKDYFPEPVTVSWNSGALTSGVHTFPAVLQSSGLYSLSSVVTVPSSSLGTQTYICNVNHKPSNTKVDKKVEPKSCDKTHTCPPCPAPEAAGGPSVFLFPPKPKDTLMISRTPEVTCVVVDVSHEDPEVKFNWYVDGVEVHNAKTKPREEQYNSTYRVVSVLTVLHQDWLNGKEYKCKVSNKALPAPIEKTISKAKGQPREPQVYTLPPSRDELTKNQVSLSCAVKGFYPSDIAVEWESNGQPENNYKTTPPVLDSDGSFFLVSKLTVDKSRWQQGNVFSCSVMHEALHNHYTQKSLSLSPGK

SEQ ID NO: 7 - protein, 687 aa, artificial sequence
EVQLVESGGGLVQPGGSLKLSCAASGFTFNTYAMNWVRDASGKGLEWVGRIRSKYNNYATYYADSVKDRFTISRDDSKSTLYLQMNSLKTEDTAVYYCARHYNFGQSYVSWFAYWGQGTTVTVSSASTKGPSVFPLAPSSKSTSGGTAALGCLVKDYFPEPVTVSWNSGALTSGVHTFPAVLQSSGLYSLSSVVTVPSSSLGTQTYICNVNHKPSNTKVDKKVEPKSCDKTHTCPPCPAPEAAGGPSVFLFPPKPKDTLMISRTPEVTCVVVDVSHEDPEVKFNWYVDGVEVHNAKTKPREEQYNSTYRVVSVLTVLHQDWLNGKEYKCKVSNKALPAPIEKTISKAKGQPREPQVYTLPPSRDELTKNQVSLSCAVKGFYPSDIAVEWESNGQPENNYKTTPPVLDSDGSFFLVSKLTVDKSRWQQGNVFSCSVMHEALHNHYTQKSLSLSPGKGGGGSGGGGSQLQLQESGPGLVKPSETLSLTCTVSGGSISSSSYYWTWIRKPPGKGLEWIGSISIAGSTYYNPSLKSRVTISVDTSKNQFSLKLSSVTAADTAVYYCARDRGDQILDVWGQGTLVTVSSASTKGPSVCPLAPSSKSTSGGTAALGCLVKDYFPEPVTVSWNSGALTSGVHTFPAVLQSSGLYSLSSVVTVPSSSLGTQTYICNVNHKPSNTKVDKKVEPKSS

SEQ ID NO: 8 - protein, 218 aa, artificial sequence
DIVMTQSPDSLAVSLGERATINCRASESVDSYGITFMNWYQDKPGQPPKLLIYAASNQGSGVPDRFSGSGSGTDFTLTISSLQAEDVAVYYCQQSKEVPWTFGQGTKLEIKRTVAAPSVFIFPPSDECLKSGTASVVCLLNNFYPREAKVQWKVDNALQSGNSQESVTEQDSKDSTYSLSSTLTLSKADYEKHKVYACEVTHQGLSSPVTKSFNRGES

SEQ ID NO: 9 - protein, 688 aa, artificial sequence
QVQLVQSGAEVKKPGASVKVSCKASGYTFIGYVMHWVRKAPGQGLEWMGYINPYNDVSQHQGKFKGRVTMTSDTSTSTVYMELSSLRSEDTAVYYCAREGRLGLRVLAYWGQGTLVTVSSASTKGPSVCPLAPSSKSTSGGTAALGCLVKDYFPEPVTVSWNSGALTSGVHTFPAVLQSSGLYSLSSVVTVPSSSLGTQTYICNVNHKPSNTKVDKKVEPKSSGGGGSGGGGSEVQLVESGGGLVQPGGSLKLSCAASGFTFNTYAMNWVRDASGKGLEWVGRIRSKYNNYATYYADSVKDRFTISRDDSKSTLYLQMNSLKTEDTAVYYCARHYNFGQSYVSWFAYWGQGTTVTVSSASTKGPSVFPLAPSSKSTSGGTAALGCLVKDYFPEPVTVSWNSGALTSGVHTFPAVLQSSGLYSLSSVVTVPSSSLGTQTYICNVNHKPSNTKVDKKVEPKSCDKTHTCPPCPAPEAAGGPSVFLFPPKPKDTLMISRTPEVTCVVVDVSHEDPEVKFNWYVDGVEVHNAKTKPREEQYNSTYRVVSVLTVLHQDWLNGKEYKCKVSNKALPAPIEKTISKAKGQPREPQVYTLPPSRDELTKNQVSLSCAVKGFYPSDIAVEWESNGQPENNYKTTPPVLDSDGSFFLVSKLTVDKSRWQQGNVFSCSVMHEALHNHYTQKSLSLSPGK

SEQ ID NO: 10 - protein, 213 aa, artificial sequence
DIQMTQSPSSLSASVGDRVTITCRASQSISRYLNWYQQKPGKAPKLLIYAASSLQSGVPSRFSGSGSGTDFTLTISSLQPEDFATYYCQQKYFDITFGGGTKVEIKRTVAAPSVFIFPPSDEQLKSGTASVVCLLNNFYPREAKVQWKVDNALQSGNSQESVTEQDSKDSTYSLSSTLTLSKADYEKHKVYACEVTHQGLSSPVTKSFNRGEC

SEQ ID NO: 11 - protein, 449 aa, artificial sequence
QLQLQESGPGLVKPSETLSLTCTVSGGSISSSSYYWTWIRQPPGKGLEWIGSISIAGSTYYNPSLKSRVTISVDTSKNQFSLKLSSVTAADTAVYYCARDRGDQILDVWGQGTLVTVSSASTKGPSVFPLAPSSKSTSGGTAALGCLVKDYFPEPVTVSWNSGALTSGVHTFPAVLQSSGLYSLSSVVTVPSSSLGTQTYICNVNHKPSNTKVDKKVEPKSCDKTHTCPPCPAPEAAGGPSVFLFPPKPKDTLMISRTPEVTCVVVDVSHEDPEVKFNWYVDGVEVHNAKTKPREEQYNSTYRVVSVLTVLHQDWLNGKEYKCKVSNKALPAPIEKTISKAKGQPREPQVYTLPPSRDELTKNQVSLWCLVKGFYPSDIAVEWESNGQPENNYKTTPPVLDSDGSFFLYSKLTVDKSRWQQGNVFSCSVMHEALHNHYTQKSLSLSPGK

SEQ ID NO: 12 - protein, 20 aa, artificial sequence
GACTCCAGAATGATGCCCCA

SEQ ID NO: 13 - protein, 20 aa, artificial sequence
CAATAACGCTGACATGTTAG

SEQ ID NO: 14 - protein, 214 aa, artificial sequence
DIQMTQSPSSLSASVGDRVTITCRASQDIRNYLNWYQQKPGKAPKLLIYYTSRLHSGVPSRFSGSGSGTDFTLTISSLQPEDFATYYCQQGNMLPWTFGQGTKLEIKRTVAAPSVFIFPPSDEQLKSGTASVVCLLNNFYPREAKVQWKVDNALQSGNSQESVTEQDSKDSTYSLSSTLTLSKADYEKHKVYACEVTHQGLSSPVTKSFNRGEC

SEQ ID NO: 15 - protein, 451 aa, artificial sequence
QVQLQESGPGLVKPSQTLSLTCTVSGYSITSDYAWNWIRQPPGKGLEWIVYIDYTGRTSYNPSLKSRVTLSRDTSKNQFSLKLSSVTAADTAVYYCARGNYGRYYYVMDYWGQGTLVTVSSASTKGPSVFPLAPSSKSTSGGTAALGCLVKDYFPEPVTVSWNSGALTSGVHTFPAVLQSSGLYSLSSVVTVPSSSLGTQTYICNVNHKPSNTKVDKKVEPKSCDKTHTCPPCPAPEAAGGPSVFLFPPKPKDTLMISRTPEVTCVVVDVSHEDPEVKFNWYVDGVEVHNAKTKPREEQYNSTYRVVSVLTVLHQDWLNGKEYKCKVSNKALPAPIEKTISKAKGQPREPQVYTLPPSRDELTKNQVSLWCLVKGFYPSDIAVEWESNGQPENNYKTTPPVLDSDGSFFLYSKLTVDKSRWQQGNVFSCSVMHEALHNHYTQKSLSLSPGK

SEQ ID NO: 16 - protein, 214 aa, artificial sequence
DIQMTQSPSSLSASVGDRVTITCRASQSISSYLNWYQQKPGKAPKLLIYAASSLQSGVPSRFSGSGSGTDFTLTISSLQPEDFATYYCQQADLPAFAFGGGTKVEIKRTVAAPSVFIFPPSDEQLKSGTASVVCLLNNFYPREAKVQWKVDNALQSGNSQESVTEQDSKDSTYSLSSTLTLSKADYEKHKVYACEVTHQGLSSPVTKSFNRGEC

SEQ ID NO: 17 - protein, 449 aa, artificial sequence
EVRLLESGGGLVQPGGSLRLSCAASGFTFSNYAMGWVRQAPGKGLEWVSAISGSGGSTYYADSVKGRFTTSRDDSKNALYLQMNSLRAEDTAVYYCARGGPGWYAADVWGQGTTVTVSSASTKGPSVFPLAPSSKSTSGGTAALGCLVKDYFPEPVTVSWNSGALTSGVHTFPAVLQSSGLYSLSSVVTVPSSSLGTQTYICNVNHKPSNTKVDKKVEPKSCDKTHTCPPCPAPEAAGGPSVFLFPPKPKDTLMISRTPEVTCVVVDVSHEDPEVKFNWYVDGVEVHNAKTKPREEQYNSTYRVVSVLTVLHQDWLNGKEYKCKVSNKALPAPIEKTISKAKGQPREPQVYTLPPSRDELTKNQVSLWCLVKGFYPSDIAVEWESNGQPENNYKTTPPVLDSDGSFFLYSKLTVDKSRWQQGNVFSCSVMHEALHNHYTQKSLSLSPGK

SEQ ID NO: 18 - protein, 214 aa, artificial sequence
DIQMTQSPSSLSASVGDRVTITCRASQSISSYLNWYQDKPGKAPKLLIYAASSLQSGVPSRFSGSGSGTDFTLTISSLQPEDFATYYCQQADLPAFAFGGGTKVEIKRTVAAPSVFIFPPSDECLKSGTASVVCLLNNFYPREAKVQWKVDNALQSGNSQESVTEQDSKDSTYSLSSTLTLSKADYEKHKVYACEVTHQGLSSPVTKSFNRGES

SEQ ID NO: 19 - protein, 7 aa, artificial sequence
HTCPXCP

SEQ ID NO: 20 - protein, 687 aa, artificial sequence
EVRLLESGGGLVQPGGSLRLSCAASGFTFSNYAMGWVRKAPGKGLEWVSAISGSGGSTYYADSVKGRFTTSRDDSKNALYLQMNSLRAEDTAVYYCARGGPGWYAADVWGQGTTVTVSSASTKGPSVCPLAPSSKSTSGGTAALGCLVKDYFPEPVTVSWNSGALTSGVHTFPAVLQSSGLYSLSSVVTVPSSSLGTQTYICNVNHKPSNTKVDKKVEPKSSGGGGSGGGGSEVQLVESGGGLVQPGGSLKLSCAASGFTFNTYAMNWVRDASGKGLEWVGRIRSKYNNYATYYADSVKDRFTISRDDSKSTLYLQMNSLKTEDTAVYYCARHGNFGQSYVSWFAYWGQGTTVTVSSASTKGPSVFPLAPSSKSTSGGTAALGCLVKDYFPEPVTVSWNSGALTSGVHTFPAVLQSSGLYSLSSVVTVPSSSLGTQTYICNVNHKPSNTKVDKKVEPKSCDKTHTCPPCPAPEAAGGPSVFLFPPKPKDTLMISRTPEVTCVVVDVSHEDPEVKFNWYVDGVEVHNAKTKPREEQYNSTYRVVSVLTVLHQDWLNGKEYKCKVSNKALPAPIEKTISKAKGQPREPQVYTLPPSRDELTKNQVSLSCAVKGFYPSDIAVEWESNGQPENNYKTTPPVLDSDGSFFLVSKLTVDKSRWQQGNVFSCSVMHEALHNHYTQKSLSLSPGK

SEQ ID NO: 21 - protein, 705 aa, artificial sequence
EVQLVESGGGLVQPGGSLKLSCAASGFTFNTYAMNWVRQASGKGLEWVGRIRSKYNNYATYYADSVKDRFTISRDDSKSTLYLQMNSLKTEDTAVYYCARHGNFGQSYVSWFAYWGQGTTVTVSSASTKGPSVFPLAPSSKSTSGGTAALGCLVKDYFPEPVTVSWNSGALTSGVHTFPAVLQSSGLYSLSSVVTVPSSSLGTQTYICNVNHKPSNTKVDKKVEPKSCDKTHTCPPCPAPEAAGGPSVFLFPPKPKDTLMISRTPEVTCVVVDVSHEDPEVKFNWYVDGVEVHNAKTKPREEQYNSTYRVVSVLTVLHQDWLNGKEYKCKVSNKALPAPIEKTISKAKGQPREPQVYTLPPSRDELTKNQVSLSCAVKGFYPSDIAVEWESNGQPENNYKTTPPVLDSDGSFFLVSKLTVDKSRWQQGNVFSCSVMHEALHNHYTQKSLSLSPGAGGGGSGGGGSDIQMTQSPSSLSASVGDRVTITCRASQSISRYLNWYQQKPGKAPKLLIYAASSLQSGVPSRFSGSGSGTDFTLTISSLQPEDFATYYCQQKYFDITFGCGTKVEIKGGGGSGGGGSGGGGSQLQLQESGPGLVKPSETLSLTCTVSGGSIVSSSYYWTWIRQPPGKCLEWIGSISIAGSTYYNPSLKSRVTISVDTSKNQFSLKLSSVTAADTAVYYCARDRGDQILDVWSQGTMVTVSS

SEQ ID NO: 22 - protein, 215 aa, artificial sequence
QAVVTQEPSLTVSPGGTVTLTCRSSTGAVTTSNYANWVQQKPGQAPRGLIGGTNKRAPGVPARFSGSLLGDKAALTLLGAQPEDEAEYYCALWYSNLWVFGQGTKLTVLGQPKAAPSVTLFPPSSEELQANKATLVCLISDFYPGAVTVAWKADSSPVKAGVETTTPSKQSNNKYAASSYLSLTPEQWKSHRSYSCQVTHEGSTVEKTVAPTECS

SEQ ID NO: 23 - protein, 705 aa, artificial sequence
EVQLVESGGGLVQPGGSLKLSCAASGFTFNTYAMNWVRQASGKGLEWVGRIRSKYNNYATYYADSVKDRFTISRDDSKSTLYLQMNSLKTEDTAVYYCARHYNFGQSYVSWFAYWGQGTTVTVSSASTKGPSVFPLAPSSKSTSGGTAALGCLVKDYFPEPVTVSWNSGALTSGVHTFPAVLQSSGLYSLSSVVTVPSSSLGTQTYICNVNHKPSNTKVDKKVEPKSCDKTHTCPPCPAPEAAGGPSVFLFPPKPKDTLMISRTPEVTCVVVDVSHEDPEVKFNWYVDGVEVHNAKTKPREEQYNSTYRVVSVLTVLHQDWLNGKEYKCKVSNKALPAPIEKTISKAKGQPREPQVYTLPPSRDELTKNQVSLSCAVKGFYPSDIAVEWESNGQPENNYKTTPPVLDSDGSFFLVSKLTVDKSRWQQGNVFSCSVMHEALHNHYTQKSLSLSPGAGGGGSGGGGSDIQMTQSPSSLSASVGDRVTITCRASQSISRYLNWYQQKPGKAPKLLIYAASSLQSGVPSRFSGSGSGTDFTLTISSLQPEDFATYYCQQKYFDITFGCGTKVEIKGGGGSGGGGSGGGGSQLQLQESGPGLVKPSETLSLTCTVSGGSIVSSSYYWTWIRQPPGKCLEWIGSISIAGSTYYNPSLKSRVTISVDTSKNQFSLKLSSVTAADTAVYYCARDRGDQILDVWSQGTMVTVSS

SEQ ID NO: 24 - protein, 125 aa, artificial sequence
EVQLVESGGGLVQPGGSLRLSCAASGFTFSNFWMTWVRQAPGKGLEWVANMNQDGSEKYYVDSVKGRFTISRDNAKSSLYLQMNSLRAEDTAVYYCARDREYCISTSCYDDFDYWGQGTLVTVSS

SEQ ID NO: 25 - protein, 108 aa, artificial sequence
DIQMTQSPSSLSASVGDRVTITCRASQSISSYLNWYQQKPGKAPKLLIYAASSLQSGVPSRFSGSGSGTDFTLTISSLQPEDFATYYCQQSYSTPPITFGQGTRLEIK

SEQ ID NO: 26 - protein, 124 aa, artificial sequence
EVQLVESGGGLVQPGRSLRLSCAASGFTFDDYSMHWVRQAPGKGLEWVSGISWNSGSKGYADSVKGRFTISRDNAKNSLYLQMNSLRAEDTALYYCAKYGSGYGKFYHYGLDVWGQGTTVTVSS

SEQ ID NO: 27 - protein, 445 aa, artificial sequence
QVQLVQSGAEVKKPGASVKVSCKASGYSFTGYTMNWVRQAPGQGLEWMGLINPYNSDTNYAQKLQGRVTMTTDTSTSTAYMELRSLRSDDTAVYYCARVALRVALDYWGQGTLVTVSSASTKGPSVFPLAPCSRSTSESTAALGCLVKDYFPEPVTVSWNSGALTSGVHTFPAVLQSSGLYSLSSVVTVPSSSLGTKTYTCNVDHKPSNTKVDKRVESKYGPPCPPCPAPEAAGGPSVFLFPPKPKDTLMISRTPEVTCVVVDVSQEDPEVQFNWYVDGVEVHNAKTKPREEQFNSTYRVVSVLTVLHQDWLNGKEYKCKVSNKGLPSSIEKTISKAKGQPREPQVYTLPPSQEEMTKNQVSLTCLVKGFYPSDIAVEWESNGQPENNYKTTPPVLDSDGSFFLYSRLTVDKSRWQEGNVFSCSVMHEALHNHYTQKSLSLSLGK

SEQ ID NO: 28 - protein, 214 aa, artificial sequence
DIQMTQSPSSLSASVGDRVTITCKASQNVATHVGWYQQKPGKAPKRLIYSASYRYSGVPSRFSGSGSGTEFTLTISNLQPEDFATYYCQQYNRYPYTFGQGTKLEIKRTVAAPSVFIFPPSDEQLKSGTASVVCLLNNFYPREAKVQWKVDNALQSGNSQESVTEQDSKDSTYSLSSTLTLSKADYEKHKVYACEVTHQGLSSPVTKSFNRGEC

SEQ ID NO: 29 - protein, 452 aa, artificial sequence
EVQLVESGGGLVQPGGSLRLSCAASGFTFNTYAMNWVRQAPGKGLEWVARIRSKYNNYATYYAASVKGRFTISRDDSKNSLYLQMNSLKTEDTAVYYCARHGNFGNSYVSWFAYWGQGTLVTVSSASTKGPSVFPLAPCSRSTSESTAALGCLVKDYFPEPVTVSWNSGALTSGVHTFPAVLQSSGLYSLSSVVTVPSSSLGTKTYTCNVDHKPSNTKVDKRVESKYGPPCPPCPAPEAAGGPSVFLFPPKPKDTLMISRTPEVTCVVVDVSQEDPEVQFNWYVDGVEVHNAKTKPREEQFNSTYRVVSVLTVLHQDWLNGKEYKCKVSNKGLPSSIEKTISKAKGQPREPQVYTLPPSQEEMTKNQVSLTCLVKGFYPSDIAVEWESNGQPENNYKTTPPVLDSDGSFLLYSKLTVDKSRWQEGNVFSCSVMHEALHNHYTQKSLSLSLGK

SEQ ID NO: 30 - protein, 215 aa, artificial sequence
QTVVTQEPSLTVSPGGTVTLTCRSSTGAVTTSNYANWVQQKPGQAPRGLIGGTNKRAPGTPARFSGSLLGGKAALTLSGVQPEDEAEYYCALWYSNLWVFGGGTKLTVLGQPKAAPSVTLFPPSSEELQANKATLVCLISDFYPGAVTVAWKADSSPVKAGVETTTPSKQSNNKYAASSYLSLTPEQWKSHRSYSCQVTHEGSTVEKTVAPTECS

SEQ ID NO: 31 - protein, 217 aa, artificial sequence
DIVLTQSPALAVSPGQRATISCRASQSVSISGINLMNWYQQKPGQQPKLLIYHASILASGIPTRFSGSGSGTDFTLTIDPVQADDIATYYCQQTRESPLTFGSGTNLEIKRTVAAPSVFIFPPSDRKLKSGTASVVCLLNNFYPREAKVQWKVDNALQSGNSQESVTEQDSKDSTYSLSSTLTLSKADYEKHKVYACEVTHQGLSSPVTKSFNRGEC

SEQ ID NO: 32 - protein, 232 aa, artificial sequence
EVQLLESGGGLVQPGGSLRLSCAASGFTFSTYAMNWVRQAPGKGLEWVSRIRSKYNNYATYYADSVKGRFTISRDDSKNTLYLQMNSLRAEDTAVYYCVRHGNFGNSYVSWFAYWGQGTLVTVSSASVAAPSVFIFPPSDEQLKSGTASVVCLLNNFYPREAKVQWKVDNALQSGNSQESVTEQDSKDSTYSLSSTLTLSKADYEKHKVYACEVTHQGLSSPVTKSFNRGEC

SEQ ID NO: 33 - protein, 447 aa, artificial sequence
ELQLEQSGGGLVQPGGSLTLSCAASGFTFSKYAMAWVRQAPTKGLEWVASISTGGVNTYYRDSVKARFTISRDNAKNTQYLQMDSLRSEDTATYYCATHTGDYFDYWGQGVMVTVSSASTKGPSVFPLAPSSKSTSGGTAALGCLVEDYFPEPVTVSWNSGALTSGVHTFPAVLQSSGLYSLSSVVTVPSSSLGTQTYICNVNHKPSNTKVDEKVEPKSCDKTHTCPPCPAPEAAGGPSVFLFPPKPKDTLMISRTPEVTCVVVDVSHEDPEVKFNWYVDGVEVHNAKTKPREEQYNSTYRVVSVLTVLHQDWLNGKEYKCKVSNKALGAPIEKTISKAKGQPREPQVCTLPPSRDELTKNQVSLSCAVKGFYPSDIAVEWESNGQPENNYKTTPPVLDSDGSFFLVSKLTVDKSRWQQGNVFSCSVMHEALHNHYTQKSLSLSPGK

SEQ ID NO: 34 - protein, 672 aa, artificial sequence
ELQLEQSGGGLVQPGGSLTLSCAASGFTFSKYAMAWVRQAPTKGLEWVASISTGGVNTYYRDSVKARFTISRDNAKNTQYLQMDSLRSEDTATYYCATHTGDYFDYWGQGVMVTVSSASTKGPSVFPLAPSSKSTSGGTAALGCLVEDYFPEPVTVSWNSGALTSGVHTFPAVLQSSGLYSLSSVVTVPSSSLGTQTYICNVNHKPSNTKVDEKVEPKSCDGGGGSGGGGSQAVVTQEPSLTVSPGGTVTLTCGSSTGAVTTSNYANWVQEKPGQAFRGLIGGTNKRAPGTPARFSGSLLGGKAALTLSGAQPEDEAEYYCALWYSNLWVFGGGTKLTVLSSASTKGPSVFPLAPSSKSTSGGTAALGCLVKDYFPEPVTVSWNSGALTSGVHTFPAVLQSSGLYSLSSVVTVPSSSLGTQTYICNVNHKPSNTKVDKKVEPKSCDKTHTCPPCPAPEAAGGPSVFLFPPKPKDTLMISRTPEVTCVVVDVSHEDPEVKFNWYVDGVEVHNAKTKPREEQYNSTYRVVSVLTVLHQDWLNGKEYKCKVSNKALGAPIEKTISKAKGQPREPQVYTLPPCRDELTKNQVSLWCLVKGFYPSDIAVEWESNGQPENNYKTTPPVLDSDGSFFLYSKLTVDKSRWQQGNVFSCSVMHEALHNHYTQKSLSLSPGK

SEQ ID NO: 35 - protein, 448 aa, artificial sequence
QLQLQESGPGLVKPSETLSLTCTVSGGSISSGSYFWGWIRQPPGKGLEWIGSIYYSGITYYNPSLKSRVTISVDTSKNQFSLKLSSVTAADTAVYYCARHDGAVAGLFDYWGQGTLVTVSSASTKGPSVFPLAPCSRSTSESTAALGCLVKDYFPEPVTVSWNSGALTSGVHTFPAVLQSSGLYSLSSVVTVPSSSLGTKTYTCNVDHKPSNTKVDKRVESKYGPPCPPCPAPEAAGGPSVFLFPPKPKDTLMISRTPEVTCVVVDVSQEDPEVQFNWYVDGVEVHNAKTKPREEQFNSTYRVVSVLTVLHQDWLNGKEYKCKVSNKGLPSSIEKTISKAKGQPREPQVYTLPPSQEEMTKNQVSLTCLVKGFYPSDIAVEWESNGQPENNYKTTPPVLDSDGSFFLYSRLTVDKSRWQEGNVFSCSVMHEALHNHYTQKSLSLSLGK

SEQ ID NO: 36 - protein, 214 aa, artificial sequence
SYVLTQPPSVSVAPGQTARITCGGNNIGSKSVHWYQQPPGQAPVVVVYDDSDRPSGIPERFSGSNSGNTATLTISRVEAGDEAVYYCQVWDSSSDHVVFGGGTKLTVLGQPKAAPSVTLFPPSSEELQANKATLVCLISDFYPGAVTVAWKGDSSPVKAGVETTTPSKQSNNKYAASSYLSLTPEQWKSHRSYSCQVTHEGSTVEKTVAPTECS

SEQ ID NO: 37 - protein, 671 aa, artificial sequence
EVQLLESGGGLVQPGGSLRLSCAASGFTFSDNAMGWVRQAPGKGLEWVSAISGPGSSTYYADSVKGRFTISRDNSKNTLYLQMNSLRAEDTAVYYCAKVLGWFDYWGQGTLVTVSSASTKGPSVFPLAPSSKSTSGGTAALGCLVEDYFPEPVTVSWNSGALTSGVHTFPAVLQSSGLYSLSSVVTVPSSSLGTQTYICNVNHKPSNTKVDEKVEPKSCDGGGGSGGGGSQAVVTQEPSLTVSPGGTVTLTCGSSTGAVTTSNYANWVQEKPGQAFRGLIGGTNKRAPGTPARFSGSLLGGKAALTLSGAQPEDEAEYYCALWYSNLWVFGGGTKLTVLSSASTKGPSVFPLAPSSKSTSGGTAALGCLVKDYFPEPVTVSWNSGALTSGVHTFPAVLQSSGLYSLSSVVTVPSSSLGTQTYICNVNHKPSNTKVDKKVEPKSCDKTHTCPPCPAPEAAGGPSVFLFPPKPKDTLMISRTPEVTCVVVDVSHEDPEVKFNWYVDGVEVHNAKTKPREEQYNSTYRVVSVLTVLHQDWLNGKEYKCKVSNKALGAPIEKTISKAKGQPREPQVYTLPPCRDELTKNQVSLWCLVKGFYPSDIAVEWESNGQPENNYKTTPPVLDSDGSFFLYSKLTVDKSRWQQGNVFSCSVMHEALHNHYTQKSLSLSPGK

SEQ ID NO: 38 - protein, 216 aa, artificial sequence
EIVLTQSPGTLSLSPGERATLSCRASQSVSDEYLSWYQQKPGQAPRLLIHSASTRATGIPDRFSGSGSGTDFTLAISRLEPEDFAVYYCQQYGYPPDFTFGQGTKVEIKRTVAAPSVFIFPPSDRKLKSGTASVVCLLNNFYPREAKVQWKVDNALQSGNSQESVTEQDSKDSTYSLSSTLTLSKADYEKHKVYACEVTHQGLSSPVTKSFNRGEC

SEQ ID NO: 39 - protein, 446 aa, artificial sequence
EVQLLESGGGLVQPGGSLRLSCAASGFTFSDNAMGWVRQAPGKGLEWVSAISGPGSSTYYADSVKGRFTISRDNSKNTLYLQMNSLRAEDTAVYYCAKVLGWFDYWGQGTLVTVSSASTKGPSVFPLAPSSKSTSGGTAALGCLVEDYFPEPVTVSWNSGALTSGVHTFPAVLQSSGLYSLSSVVTVPSSSLGTQTYICNVNHKPSNTKVDEKVEPKSCDKTHTCPPCPAPEAAGGPSVFLFPPKPKDTLMISRTPEVTCVVVDVSHEDPEVKFNWYVDGVEVHNAKTKPREEQYNSTYRVVSVLTVLHQDWLNGKEYKCKVSNKALGAPIEKTISKAKGQPREPQVCTLPPSRDELTKNQVSLSCAVKGFYPSDIAVEWESNGQPENNYKTTPPVLDSDGSFFLVSKLTVDKSRWQQGNVFSCSVMHEALHNHYTQKSLSLSPGK

SEQ ID NO: 40 - protein, 121 aa, artificial sequence
QVQLQESGPGLVKPSQTLSLTCTVSGYSITSDYAWNWIRQPPGKGLEWIVYIDYTGRTSYNPSLKSRVTLSRDTSKNQFSLKLSSVTAADTAVYYCARGNYGRYYYVMDYWGQGTLVTVSS

SEQ ID NO: 41 - protein, 6 aa, artificial sequence
SDYAWN

SEQ ID NO: 42 - protein, 16 aa, artificial sequence
YIDYTGRTSYNPSLKS

SEQ ID NO: 43 - protein, 12 aa, artificial sequence
GNYGRYYYVMDY

SEQ ID NO: 44 - protein, 107 aa, artificial sequence
DIQMTQSPSSLSASVGDRVTITCRASQDIRNYLNWYQQKPGKAPKLLIYYTSRLHSGVPSRFSGSGSGTDFTLTISSLQPEDFATYYCQQGNMLPWTFGQGTKLEIK

SEQ ID NO: 45 - protein, 11 aa, artificial sequence
RASQDIRNYLN

SEQ ID NO: 46 - protein, 7 aa, artificial sequence
YTSRLHS

SEQ ID NO: 47 - protein, 9 aa, artificial sequence
QQGNMLPWT

SEQ ID NO: 48 - protein, 120 aa, artificial sequence
QVQLVQSGAEVKKPGASVKVSCKASGYTFIGYVMHWVRQAPGQGLEWMGYINPYNDVSQHQGKFKGRVTMTSDTSTSTVYMELSSLRSEDTAVYYCAREGRLGLRVLAYWGQGTLVTVSS

SEQ ID NO: 49 - protein, 5 aa, artificial sequence
GYVMH

SEQ ID NO: 50 - protein, 17 aa, artificial sequence
YINPYNDVSQHQGKFKG

SEQ ID NO: 51 - protein, 11 aa, artificial sequence
EGRLGLRVLAY

SEQ ID NO: 52 - protein, 111 aa, artificial sequence
DIVMTQSPDSLAVSLGERATINCRASESVDSYGITFMNWYQQKPGQPPKLLIYAASNQGSGVPDRFSGSGSGTDFTLTISSLQAEDVAVYYCQQSKEVPWTFGQGTKLEIK

SEQ ID NO: 53 - protein, 15 aa, artificial sequence
RASESVDSYGITFMN

SEQ ID NO: 54 - protein, 7 aa, artificial sequence
AASNQGS

SEQ ID NO: 55 - protein, 9 aa, artificial sequence
QQSKEVPWT

SEQ ID NO: 56 - protein, 119 aa, artificial sequence
QLQLQESGPGLVKPSETLSLTCTVSGGSISSSSYYWTWIRQPPGKGLEWIGSISIAGSTYYNPSLKSRVTISVDTSKNQFSLKLSSVTAADTAVYYCARDRGDQILDVWGQGTLVTVSS

SEQ ID NO: 57 - protein, 7 aa, artificial sequence
SSSYYWT

SEQ ID NO: 58 - protein, 16 aa, artificial sequence
SISIAGSTYYNPSLKS

SEQ ID NO: 59 - protein, 9 aa, artificial sequence
DRGDQILDV

SEQ ID NO: 60 - protein, 106 aa, artificial sequence
DIQMTQSPSSLSASVGDRVTITCRASQSISRYLNWYQQKPGKAPKLLIYAASSLQSGVPSRFSGSGSGTDFTLTISSLQPEDFATYYCQQKYFDITFGGGTKVEIK

SEQ ID NO: 61 - protein, 11 aa, artificial sequence
RASQSISRYLN

SEQ ID NO: 62 - protein, 7 aa, artificial sequence
AASSLQS

SEQ ID NO: 63 - protein, 8 aa, artificial sequence
QQKYFDIT

SEQ ID NO: 64 - protein, 125 aa, artificial sequence
EVQLVESGGGLVQPGGSLKLSCAASGFTFNTYAMNWVRQASGKGLEWVGRIRSKYNNYATYYADSVKDRFTISRDDSKSTLYLQMNSLKTEDTAVYYCARHGNFGQSYVSWFAYWGQGTTVTVSS

SEQ ID NO: 65 - protein, 5 aa, artificial sequence
TYAMN

SEQ ID NO: 66 - protein, 19 aa, artificial sequence
RIRSKYNNYATYYADSVKD

SEQ ID NO: 67 - protein, 14 aa, artificial sequence
HGNFGQSYVSWFAY

SEQ ID NO: 68 - protein, 109 aa, artificial sequence
QAVVTQEPSLTVSPGGTVTLTCRSSTGAVTTSNYANWVQQKPGQAPRGLIGGTNKRAPGVPARFSGSLLGDKAALTLLGAQPEDEAEYYCALWYSNLWVFGQGTKLTVL

SEQ ID NO: 69 - protein, 14 aa, artificial sequence
RSSTGAVTTSNYAN

SEQ ID NO: 70 - protein, 7 aa, artificial sequence
GTNKRAP

SEQ ID NO: 71 - protein, 9 aa, artificial sequence
ALWYSNLWV

SEQ ID NO: 72 - protein, 125 aa, artificial sequence
EVQLVESGGGLVQPGGSLKLSCAASGFTFNTYAMNWVRQASGKGLEWVGRIRSKYNNYATYYADSVKDRFTISRDDSKSTLYLQMNSLKTEDTAVYYCARHYNFGQSYVSWFAYWGQGTTVTVSS

SEQ ID NO: 73 - protein, 14 aa, artificial sequence
HYNFGQSYVSWFAY

SEQ ID NO: 74 - protein, 109 aa, artificial sequence
QAVVTQEPSLTVSPGGTVTLTCRSSTGAVTTSNYANWVQKKPGQAPRGLIGGTNKRAPGVPARFSGSLLGDKAALTLLGAQPEDEAEYYCALWYSNLWVFGQGTKLTVL

SEQ ID NO: 75 - protein, 106 aa, artificial sequence
DIQMTQSPSSLSASVGDRVTITCRASQSISRYLNWYQDKPGKAPKLLIYAASSLQSGVPSRFSGSGSGTDFTLTISSLQPEDFATYYCQQKYFDITFGGGTKVEIK

SEQ ID NO: 76 - protein, 119 aa, artificial sequence
QLQLQESGPGLVKPSETLSLTCTVSGGSISSSSYYWTWIRKPPGKGLEWIGSISIAGSTYYNPSLKSRVTISVDTSKNQFSLKLSSVTAADTAVYYCARDRGDQILDVWGQGTLVTVSS

SEQ ID NO: 77 - protein, 125 aa, artificial sequence
EVQLVESGGGLVQPGGSLKLSCAASGFTFNTYAMNWVRDASGKGLEWVGRIRSKYNNYATYYADSVKDRFTISRDDSKSTLYLQMNSLKTEDTAVYYCARHGNFGQSYVSWFAYWGQGTTVTVSS

SEQ ID NO: 78 - protein, 125 aa, artificial sequence
EVQLVESGGGLVQPGGSLKLSCAASGFTFNTYAMNWVRDASGKGLEWVGRIRSKYNNYATYYADSVKDRFTISRDDSKSTLYLQMNSLKTEDTAVYYCARHYNFGQSYVSWFAYWGQGTTVTVSS

SEQ ID NO: 79 - protein, 111 aa, artificial sequence
DIVMTQSPDSLAVSLGERATINCRASESVDSYGITFMNWYQDKPGQPPKLLIYAASNQGSGVPDRFSGSGSGTDFTLTISSLQAEDVAVYYCQQSKEVPWTFGQGTKLEIK

SEQ ID NO: 80 - protein, 120 aa, artificial sequence
QVQLVQSGAEVKKPGASVKVSCKASGYTFIGYVMHWVRKAPGQGLEWMGYINPYNDVSQHQGKFKGRVTMTSDTSTSTVYMELSSLRSEDTAVYYCAREGRLGLRVLAYWGQGTLVTVSS

SEQ ID NO: 81 - protein, 5 aa, artificial sequence
CPXCP

SEQ ID NO: 82 - protein, 103 aa, artificial sequence
ASTKGPSVFPLAPSSKSTSGGTAALGCLVKDYFPEPVTVSWNSGALTSGVHTFPAVLQSSGLYSLSSVVTVPSSSLGTQTYICNVNHKPSNTKVDKKVEPKSC

SEQ ID NO: 83 - protein, 110 aa, artificial sequence
APELLGGPSVFLFPPKPKDTLMISRTPEVTCVVVDVSHEDPEVKFNWYVDGVEVHNAKTKPREEQYNSTYRVVSVLTVLHQDWLNGKEYKCKVSNKALPAPIEKTISKAK

SEQ ID NO: 84 - protein, 107 aa, artificial sequence
GQPREPQVYTLPPSRDELTKNQVSLTCLVKGFYPSDIAVEWESNGQPENNYKTTPPVLDSDGSFFLYSKLTVDKSRWQQGNVFSCSVMHEALHNHYTQKSLSLSPGK

SEQ ID NO: 85 - protein, 103 aa, artificial sequence
ASTKGPSVCPLAPSSKSTSGGTAALGCLVKDYFPEPVTVSWNSGALTSGVHTFPAVLQSSGLYSLSSVVTVPSSSLGTQTYICNVNHKPSNTKVDKKVEPKSC

SEQ ID NO: 86 - protein, 103 aa, artificial sequence
ASTKGPSVCPLAPSSKSTSGGTAALGCLVKDYFPEPVTVSWNSGALTSGVHTFPAVLQSSGLYSLSSVVTVPSSSLGTQTYICNVNHKPSNTKVDKKVEPKSS

SEQ ID NO: 87 - protein, 227 aa, artificial sequence
DKTHTCPPCPAPELLGGPSVFLFPPKPKDTLMISRTPEVTCVVVDVSHEDPEVKFNWYVDGVEVHNAKTKPREEQYNSTYRVVSVLTVLHQDWLNGKEYKCKVSNKALPAPIEKTISKAKGQPREPQVYTLPPSRDELTKNQVSLTCLVKGFYPSDIAVEWESNGQPENNYKTTPPVLDSDGSFFLYSKLTVDKSRWQQGNVFSCSVMHEALHNHYTQKSLSLSPGK

SEQ ID NO: 88 - protein, 224 aa, artificial sequence
PPCPSCPAPEFLGGPSVFLFPPKPKDTLMISRTPEVTCVVVDVSQEDPEVQFNWYVDGVEVHNAKTKPREEQFNSTYRVVSVLTVLHQDWLNGKEYKCKVSNKGLPSSIEKTISKAKGQPREPQVYTLPPSQEEMTKNQVSLTCLVKGFYPSDIAVEWESNGQPENNYKTTPPVLDSDGSFFLYSRLTVDKSRWQEGNVFSCSVMHEALHNHYTQKSLSLSLGK

SEQ ID NO: 89 - protein, 227 aa, artificial sequence
DKTHTCPPCPAPEAAGGPSVFLFPPKPKDTLMISRTPEVTCVVVDVSHEDPEVKFNWYVDGVEVHNAKTKPREEQYNSTYRVVSVLTVLHQDWLNGKEYKCKVSNKALPAPIEKTISKAKGQPREPQVYTLPPSRDELTKNQVSLTCLVKGFYPSDIAVEWESNGQPENNYKTTPPVLDSDGSFFLYSKLTVDKSRWQQGNVFSCSVMHEALHNHYTQKSLSLSPGK

SEQ ID NO: 90 - protein, 224 aa, artificial sequence
PPCPSCPAPEAAGGPSVFLFPPKPKDTLMISRTPEVTCVVVDVSQEDPEVQFNWYVDGVEVHNAKTKPREEQFNSTYRVVSVLTVLHQDWLNGKEYKCKVSNKGLPSSIEKTISKAKGQPREPQVYTLPPSQEEMTKNQVSLTCLVKGFYPSDIAVEWESNGQPENNYKTTPPVLDSDGSFFLYSRLTVDKSRWQEGNVFSCSVMHEALHNHYTQKSLSLSLGK

SEQ ID NO: 91 - protein, 227 aa, artificial sequence
DKTHTCPPCPAPELLGGPSVFLFPPKPKDTLMISRTPEVTCVVVDVSHEDPEVKFNWYVDGVEVHNAKTKPREEQYNSTYRVVSVLTVLHQDWLNGKEYKCKVSNKALPAPIEKTISKAKGQPREPQVYTLPPSRDELTKNQVSLSCAVKGFYPSDIAVEWESNGQPENNYKTTPPVLDSDGSFFLVSKLTVDKSRWQQGNVFSCSVMHEALHNHYTQKSLSLSPGK

SEQ ID NO: 92 - protein, 227 aa, artificial sequence [sequence omitted]

SEQ ID NO: 93 - protein, 227 aa, artificial sequence
DKTHTCPPCPAPEAAGGPSVFLFPPKPKDTLMISRTPEVTCVVVDVSHEDPEVKFNWYVDGVEVHNAKTKPREEQYNSTYRVVSVLTVLHQDWLNGKEYKCKVSNKALPAPIEKTISKAKGQPREPQVYTLPPSRDELTKNQVSLSCAVKGFYPSDIAVEWESNGQPENNYKTTPPVLDSDGSFFLVSKLTVDKSRWQQGNVFSCSVMHEALHNHYTQKSLSLSPGK

SEQ ID NO: 94 - protein, 227 aa, artificial sequence
DKTHTCPPCPAPEAAGGPSVFLFPPKPKDTLMISRTPEVTCVVVDVSHEDPEVKFNWYVDGVEVHNAKTKPREEQYNSTYRVVSVLTVLHQDWLNGKEYKCKVSNKALPAPIEKTISKAKGQPREPQVYTLPPSRDELTKNQVSLWCLVKGFYPSDIAVEWESNGQPENNYKTTPPVLDSDGSFFLYSKLTVDKSRWQQGNVFSCSVMHEALHNHYTQKSLSLSPGK

SEQ ID NO: 95 - protein, 107 aa, artificial sequence [sequence omitted]

SEQ ID NO: 96 - protein, 106 aa, artificial sequence
GQPKAAPSVTLFPPSSEELQANKATLVCLISDFYPGAVTVAWKADSSPVKAGVETTTPSKQSNNKYAASSYLSLTPEQWKSHRSYSCQVTHEGSTVEKTVAPTECS

SEQ ID NO: 97 - protein, 107 aa, artificial sequence
RTVAAPSVFIFPPSDECLKSGTASVVCLLNNFYPREAKVQWKVDNALQSGNSQESVTEQDSKDSTYSLSSTLTLSKADYEKHKVYACEVTHQGLSSPVTKSFNRGEC

SEQ ID NO: 98 - protein, 107 aa, artificial sequence
RTVAAPSVFIFPPSDECLKSGTASVVCLLNNFYPREAKVQWKVDNALQSGNSQESVTEQDSKDSTYSLSSTLTLSKADYEKHKVYACEVTHQGLSSPVTKSFNRGES

SEQ ID NO: 99 - protein, 10 aa, artificial sequence
DKTHTCPXCP

SEQ ID NO: 100 - protein, 214 aa, artificial sequence; identical to SEQ ID NO: 16

SEQ ID NO: 101 - protein, 449 aa, artificial sequence
EVRLLESGGGLVQPGGSLRLSCAASGFTFSNYAMGWVRQAPGKGLEWVSAISGSGGSTYYADSVKGRFTTSRDDSKNALYLQMNSLRAEDTAVYYCARGGPGWYAADVWGQGTTVTVSSASTKGPSVFPLAPSSKSTSGGTAALGCLVKDYFPEPVTVSWNSGALTSGVHTFPAVLQSSGLYSLSSVVTVPSSSLGTQTYICNVNHKPSNTKVDKKVEPKSCDKTHTCPPCPAPEAAGGPSVFLFPPKPKDTLMISRTPEVTCVVVDVSHEDPEVKFNWYVDGVEVHNAKTKPREEQYNSTYRVVSVLTVLHQDWLNGKEYKCKVSNKALPAPIEKTISKAKGQPREPQVYTLPPSRDELTKNQVSLTCLVKGFYPSDIAVEWESNGQPENNYKTTPPVLDSDGSFFLYSKLTVDKSRWQQGNVFSCSVMHEALHNHYTQKSLSLSPGK

SEQ ID NO: 102 - protein, 184 aa, artificial sequence
MLQMAGQCSQNEYFDSLLHACIPCQLRCSSNTPPLTCQRYCNASVTNSVKGTNAILWTCLGLSLIISLAVFVLMFLLRKINSEPLKDEFKNTGSGLLGMANIDLEKSRTGDEIILPRGLEYTVEECTCEDCIKSKPKVDSDHCFPLPAMEEGATILVTTKTNDYCKSLPAALSATEIEKSISAR

SEQ ID NO: 103 - protein, 183 aa, artificial sequence
MLQMAGQCSQNEYFDSLLHACIPCQLRCSSNTPLTCQRYCNASVTNSVKGTNAILWTCLGLSLIISLAVFVLMFLLRKINSEPLKDEFKNTGSGLLGMANIDLEKSRTGDEIILPRGLEYTVEECTCEDCIKSKPKVDSDHCFPLPAMEEGATILVTTKTNDYCKSLPAALSATEIEKSISAR

SEQ ID NO: 104 - protein, 184 aa, artificial sequence
MLQMAGQCSQNEYFDSLLHACIPCQLPCSSNTPPLTCQRYCNASVTNSVKGTNAILWTCLGLSLIISLAVFVLMFLLRKINSEPLKDEFKNTGSGLLGMANIDLEKSRTGDEIILPRGLEYTVEECTCEDCIKSKPKVDSDHCFPLPAMEEGATILVTTKTNDYCKSLPAALSATEIEKSISAR

SEQ ID NO: 105 - protein, 184 aa, artificial sequence
MLQMAGQCSQNEYFDSLLHACIPCQLRCSSNTPPLTCQAYCNASVTNSVKGTNAILWTCLGLSLIISLAVFVLMFLLRKINSEPLKDEFKNTGSGLLGMANIDLEKSRTGDEIILPRGLEYTVEECTCEDCIKSKPKVDSDHCFPLPAMEEGATILVTTKTNDYCKSLPAALSATEIEKSISAR

SEQ ID NO: 106 - protein, 183 aa, artificial sequence
MLQMAGQCSQNEYFDSLLHACIPCQLRCSNTPPLTCQRYCNASVTNSVKGTNAILWTCLGLSLIISLAVFVLMFLLRKINSEPLKDEFKNTGSGLLGMANIDLEKSRTGDEIILPRGLEYTVEECTCEDCIKSKPKVDSDHCFPLPAMEEGATILVTTKTNDYCKSLPAALSATEIEKSISAR

SEQ ID NO: 107 - DNA, 552 bp, artificial sequence
  source 1..552: mol_type = other DNA
atgttgcagatggctgggcagtgctcccaaaatgaatattttgacagtttgttgcatgcttgcataccttgtcaacttcgatgttcttctaatactcctcctctaacatgtcagcgttattgtaatgcaagtgtgaccaattcagtgaaaggaacgaatgcgattctctggacctgtttgggactgagcttaataatttctttggcagttttcgtgctaatgtttttgctaaggaagataaactctgaaccattaaaggacgagtttaaaaacacaggatcaggtctcctgggcatggctaacattgacctggaaaagagcaggactggtgatgaaattattcttccgagaggcctcgagtacacggtggaagaatgcacctgtgaagactgcatcaagagcaaaccgaaggtggactctgaccattgctttccactcccagctatggaggaaggcgcaaccattcttgtcaccacgaaaacgaatgactattgcaagagcctgccagctgctttgagtgctacggagatagagaaatcaatttctgctagg

SEQ ID NO: 108 - DNA, 549 bp, artificial sequence
  source 1..549: mol_type = other DNA
atgttgcagatggctgggcagtgctcccaaaatgaatattttgacagtttgttgcatgcttgcataccttgtcaacttcgatgttcttctaatactcctctaacatgtcagcgttattgtaatgcaagtgtgaccaattcagtgaaaggaacgaatgcgattctctggacctgtttgggactgagcttaataatttctttggcagttttcgtgctaatgtttttgctaaggaagataaactctgaaccattaaaggacgagtttaaaaacacaggatcaggtctcctgggcatggctaacattgacctggaaaagagcaggactggtgatgaaattattcttccgagaggcctcgagtacacggtggaagaatgcacctgtgaagactgcatcaagagcaaaccgaaggtggactctgaccattgctttccactcccagctatggaggaaggcgcaaccattcttgtcaccacgaaaacgaatgactattgcaagagcctgccagctgctttgagtgctacggagatagagaaatcaatttctgctagg

SEQ ID NO: 109 - DNA, 552 bp, artificial sequence
  source 1..552: mol_type = other DNA
atgttgcagatggctgggcagtgctcccaaaatgaatattttgacagtttgttgcatgcttgcataccttgtcaacttccttgttcttctaatactcctcctctaacatgtcagcgttattgtaatgcaagtgtgaccaattcagtgaaaggaacgaatgcgattctctggacctgtttgggactgagcttaataatttctttggcagttttcgtgctaatgtttttgctaaggaagataaactctgaaccattaaaggacgagtttaaaaacacaggatcaggtctcctgggcatggctaacattgacctggaaaagagcaggactggtgatgaaattattcttccgagaggcctcgagtacacggtggaagaatgcacctgtgaagactgcatcaagagcaaaccgaaggtggactctgaccattgctttccactcccagctatggaggaaggcgcaaccattcttgtcaccacgaaaacgaatgactattgcaagagcctgccagctgctttgagtgctacggagatagagaaatcaatttctgctagg

SEQ ID NO: 110 - DNA, 552 bp, artificial sequence
  source 1..552: mol_type = other DNA
atgttgcagatggctgggcagtgctcccaaaatgaatattttgacagtttgttgcatgcttgcataccttgtcaacttcgatgttcttctaatactcctcctctaacatgtcaggcttattgtaatgcaagtgtgaccaattcagtgaaaggaacgaatgcgattctctggacctgtttgggactgagcttaataatttctttggcagttttcgtgctaatgtttttgctaaggaagataaactctgaaccattaaaggacgagtttaaaaacacaggatcaggtctcctgggcatggctaacattgacctggaaaagagcaggactggtgatgaaattattcttccgagaggcctcgagtacacggtggaagaatgcacctgtgaagactgcatcaagagcaaaccgaaggtggactctgaccattgctttccactcccagctatggaggaaggcgcaaccattcttgtcaccacgaaaacgaatgactattgcaagagcctgccagctgctttgagtgctacggagatagagaaatcaatttctgctagg

SEQ ID NO: 111 - DNA, 549 bp, artificial sequence
  source 1..549: mol_type = other DNA
atgttgcagatggctgggcagtgctcccaaaatgaatattttgacagtttgttgcatgcttgcataccttgtcaacttcgatgttctaatactcctcctctaacatgtcagcgttattgtaatgcaagtgtgaccaattcagtgaaaggaacgaatgcgattctctggacctgtttgggactgagcttaataatttctttggcagttttcgtgctaatgtttttgctaaggaagataaactctgaaccattaaaggacgagtttaaaaacacaggatcaggtctcctgggcatggctaacattgacctggaaaagagcaggactggtgatgaaattattcttccgagaggcctcgagtacacggtggaagaatgcacctgtgaagactgcatcaagagcaaaccgaaggtggactctgaccattgctttccactcccagctatggaggaaggcgcaaccattcttgtcaccacgaaaacgaatgactattgcaagagcctgccagctgctttgagtgctacggagatagagaaatcaatttctgctagg

SEQ ID NO: 112 - skipped

SEQ ID NO: 113 - protein, 5 aa, synthetic construct
  REPEAT 1..5: note = Repeated for at least 1 time, preferably 2, 3, 4, 5, 6, 7, 8, 9 or 10 times
GSGGS

SEQ ID NO: 114 - protein, 5 aa, synthetic construct
  REPEAT 1..5: note = Repeated for at least 1 time, preferably 2, 3, 4, 5, 6, 7, 8, 9 or 10 times
GGGGS

SEQ ID NO: 115 - protein, 4 aa, synthetic construct
  REPEAT 1..4: note = Repeated for at least 1 time, preferably 2, 3, 4, 5, 6, 7, 8, 9 or 10 times
GGGS

SEQ ID NO: 116 - protein, 6 aa, synthetic construct
  REPEAT 1..5: note = Repeated for at least 1 time, preferably 2, 3, 4, 5, 6, 7, 8, 9 or 10 times
GGGGSG